European Patent Application EP 4 733 393 A1, published April 29, 2026. Title: Immunostimulatory Herpesvirus. Applicant: The University of Tokyo. The sequence listing filed with the application follows.

SEQUENCE LISTING (32 sequences)

SEQ ID NO: 1 - protein, 21 aa, synthetic construct
METDTLLLWVLLLWVPGSTGD

SEQ ID NO: 2 - protein, 4 aa, synthetic construct
AAQP

SEQ ID NO: 3 - protein, 121 aa, Armecian hamster
EVRLLESGGGLVKPEGSLKLSCVASGFTFSDYFMSWVRQAPGKGLEWVAHIYTKSYNYATYYSGSVKGRFTISRDDSRSMVYLQMNNLRTEDTATYYCTRDGSGYPSLDFWGQGTQVTVSS

SEQ ID NO: 4 - protein, 327 aa, Homo sapiens
ASTKGPSVFPLAPCSRSTSESTAALGCLVKDYFPEPVTVSWNSGALTSGVHTFPAVLQSSGLYSLSSVVTVPSSSLGTKTYTCNVDHKPSNTKVDKRVESKYGPPCPPCPAPEFLGGPSVFLFPPKPKDTLMISRTPEVTCVVVDVSQEDPEVQFNWYVDGVEVHNAKTKPREEQFNSTYRVVSVLTVLHQDWLNGKEYKCKVSNKGLPSSIEKTISKAKGQPREPQVYTLPPSQEEMTKNQVSLTCLVKGFYPSDIAVEWESNGQPENNYKTTPPVLDSDGSFFLYSRLTVDKSRWQEGNVFSCSVMHEALHNHYTQKSLSLSLGK

SEQ ID NO: 5 - protein, 4 aa, synthetic construct
RKRR

SEQ ID NO: 6 - protein, 24 aa, synthetic construct
APVKQTLNFDLLKLAGDVESNPGP

SEQ ID NO: 7 - protein, 108 aa, Armecian hamster
YELTQPPSASVVGETVKITCSGDQLPKYFADWFHQRSDQTILQVIYDDNKRPSGIPERISGSSSGTTATLTIRDVRAEDEGDYYCFSGYVDSDSKLYVFGSGTQLTVL

SEQ ID NO: 8 - protein, 106 aa, Homo sapiens
GQPKAAPSVTLFPPSSEELQANKATLVCLISDFYPGAVTVAWKADSSPVKAGVETTTPSKQSNNKYAASSYLSLTPEQWKSHRSYSCQVTHEGSTVEKTVAPTECS

SEQ ID NO: 9 - protein, 350 aa, Armecian hamster
YWGQGTMVAVSSATTTAPSVYPLAPACDSTTSTTDTVTLGCLVKGYFPEPVTVSWNSGALTSGVHTFPSVLHSGLYSLSSSVTVPSSTWPKQPITCNVAHPASSTKVDKKIEPRTDTDTCPNPPDPCPTCPTPDLLGGPSVFIFPPKPKDVLMISLTPKITCVVVDVSEEEPDVQFNWYVNNVEDKTAQTETRQRQYNSTYRVVSVLPIKHQDWMSGKVFKCKVNNNALPSPIEKTISKPRGQVRVPQIYTFPPPIEQTVKKDVSVTCLVTGFLPQDIHVEWESNGQPQPEQNYKNTQPVLDSDGSYFLYSKLNVPKSRWDQGDSFTCSVIHEALHNHHMTKTISRSLGN

SEQ ID NO: 10 - protein, 110 aa, Armecian hamster
EIKRADAKPTVSIFPPSSEQLGTGSATLVCFVNNFYPKDINVKWKVDGSEKRDGVLQSVTDQDSKDSTYSLSSTLSLTKADYERHNLYTCEVTHKTSTAAIVKTLNRNEC

SEQ ID NO: 11 - protein, 118 aa, synthetic construct [sequence omitted]

SEQ ID NO: 12 - protein, 330 aa, Homo sapiens
ASTKGPSVFPLAPSSKSTSGGTAALGCLVKDYFPEPVTVSWNSGALTSGVHTFPAVLQSSGLYSLSSVVTVPSSSLGTQTYICNVNHKPSNTKVDKKVEPKSCDKTHTCPPCPAPELLGGPSVFLFPPKPKDTLMISRTPEVTCVVVDVSHEDPEVKFNWYVDGVEVHNAKTKPREEQYASTYRVVSVLTVLHQDWLNGKEYKCKVSNKALPAPIEKTISKAKGQPREPQVYTLPPSREEMTKNQVSLTCLVKGFYPSDIAVEWESNGQPENNYKTTPPVLDSDGSFFLYSKLTVDKSRWQQGNVFSCSVMHEALHNHYTQKSLSLSPGK

SEQ ID NO: 13 - protein, 108 aa, synthetic construct
DIQMTQSPSSLSASVGDRVTITCRASQDVSTAVAWYQQKPGKAPKLLIYSASFLYSGVPSRFSGSGSGTDFTLTISSLQPEDFATYYCQQYLYHPATFGQGTKVEIKR

SEQ ID NO: 14 - protein, 105 aa, Homo sapiens
TVAAPSVFIFPPSDEQLKSGTASVVCLLNNFYPREAKVQWKVAALQSGNSQESVTEQDSKDSTYSLSSTLTLSKADYEKHKVYACEVTHQGLSSPVTKSFNRGEC

SEQ ID NO: 15 - protein, 134 aa, synthetic construct
GWSWIILFLVTAATGVHTQVQLLQSESELVKPGASVKLSCKTSGYTFTDYYIHWVKQKPGQGLEWIGLINPNNDGTNYNQKFQGKATLTADKSSSTAYMELNSLTFDDSVIYFCARASSRLRMARTTSDYYAMD

SEQ ID NO: 16 - protein, 330 aa, Homo sapiens
ASTKGPSVFPLAPSSKSTSGGTAALGCLVKDYFPEPVTVSWNSGALTSGVHTFPAVLQSSGLYSLSSVVTVPSSSLGTQTYICNVNHKPSNTKVDKKVEPKSCDKTHTCPPCPAPELLGGPSVFLFPPKPKDTLMISRTPEVTCVVVDVSHEDPEVKFNWYVDGVEVHNAKTKPREEQYNSTYRVVSVLTVLHQDWLNGKEYKCKVSNKALPAPIEKTISKAKGQPREPQVYTLPPSRDELTKNQVSLTCLVKGFYPSDIAVEWESNGQPENNYKTTPPVLDSDGSFFLYSKLTVDKSRWQQGNVFSCSVMHEGLHNHYTQKSLSLSPGK

SEQ ID NO: 17 - protein, 139 aa, synthetic construct
GEHHQTDRGSNMESHTQALMSLLLWISGACADIVMTQSPSSLAVSVGEKVTISCKSSQSLLYGSSHYLAWYQQKVGQSPKLLIYWASTRHTGIPDRFIGSGSGTDFTLSLSSVQAEDMADYFCQQYFSTPWTFGAGTRV

SEQ ID NO: 18 - protein, 121 aa, synthetic construct
RLLGLLYLVTALPGVLSQIQLQESGPGLVNPSQSLSLSCSVTGYSITSGYGWNWIRQFPGQKVEWMGFIYYEGSTYYNPSIKSRISITRDTSKNQFFLQVNSVTTEDTATYYCARQTGYFD

SEQ ID NO: 19 - protein, 129 aa, synthetic construct
ESHIHVFMSLFLWVSGSCADIMMTQSPSSLSVSAGEKATISCKSSQSLFNSNAKTNYLNWYLQKPGQSPKLLIYYASTRHTGVPDRFRGSGSGTDFTLTISSVQDEDLAFYYCQQWYDYPYTFGAGTKV

SEQ ID NO: 20 - protein, 103 aa, synthetic construct
IQLQESGPGLVNPSQSLSLSCSVTGYSITSGYGWNWIRQFPGQKVEWMGFIYYEGSTYYNPSIKSRISITRDTSKNQFFLQVNSVTTEDTATYYCARQTGYFD

SEQ ID NO: 21 - protein, 110 aa, synthetic construct
DIMMTQSPSSLSVSAGEKATISCKSSQSLFNSNAKTNYLNWYLQKPGQSPKLLIYYASTRHTGVPDRFRGSGSGTDFTLTISSVQDEDLAFYYCQQWYDYPYTFGAGTKV

SEQ ID NO: 22 - protein, 113 aa, synthetic construct [sequence omitted]

SEQ ID NO: 23 - protein, 327 aa, Homo sapiens; identical to SEQ ID NO: 4

SEQ ID NO: 24 - protein, 108 aa, synthetic construct
EIVLTQSPATLSLSPGERATLSCRASQSVSSYLAWYQQKPGQAPRLLIYDASNRATGIPARFSGSGSGTDFTLTISSLEPEDFAVYYCQQSSNWPRTFGQGTKVEIKR

SEQ ID NO: 25 - protein, 118 aa, synthetic construct
QVQLVESGGGVVQPGRSLRLSCAASGFTFSSYTMHWVRQAPGKGLEWVTSISYDGNNKYYADSVKGRFTISRDNSKNTLYLQMNSLRAEDTAIYYCARTGWLGPFDYWGQGTLVTVSS

SEQ ID NO: 26 - protein, 109 aa, synthetic construct
EIVLTQSPGTLSLSPGERATLSCRASQSVGSSYLAWYQQKPGQAPRLLIYGAFSRATGIPDRFSGSGSGTDFTLTISRLEPEDFAVYYCQQYGSSPWTFGQGTKVEIKR

SEQ ID NO: 27 - protein, 125 aa, synthetic construct
QVQLVESGGGVVQPGRSLRLSCAASGFTFSSYGMHWVRQAPGKGLEWVAVIWYDGSNKYYADSVKGRFTISRDNSKNTLYLQMNSLRAEDTAVYYCARDPRGATLYYYYYGMDVWGQGTTVTVSS

SEQ ID NO: 28 - protein, 326 aa, Homo sapiens
ASTKGPSVFPLAPCSRSTSESTAALGCLVKDYFPEPVTVSWNSGALTSGVHTFPAVLQSSGLYSLSSVVTVPSSNFGTQTYTCNVDHKPSNTKVDKTVERKCCVECPPCPAPPVAGPSVFLFPPKPKDTLMISRTPEVTCVVVDVSHEDPEVQFNWYVDGVEVHNAKTKPREEQFNSTFRVVSVLTVVHQDWLNGKEYKCKVSNKGLPAPIEKTISKTKGQPREPQVYTLPPSREEMTKNQVSLTCLVKGFYPSDISVEWESNGQPENNYKTTPPMLDSDGSFFLYSKLTVDKSRWQQGNVFSCSVMHEALHNHYTQKSLSLSPGK

SEQ ID NO: 29 - protein, 108 aa, synthetic construct
DIQMTQSPSSLSASVGDRVTITCRASQSINSYLDWYQQKPGKAPKLLIYAASSLQSGVPSRFSGSGSGTDFTLTISSLQPEDFATYYCQQYYSTPFTFGPGTKVEIKR

SEQ ID NO: 30 - DNA, 10156 bp, synthetic construct
  source 1..10156: mol_type = other DNA
accacaggtgggtgctttggaaacttgtcggtcgccgtgctcctgtgagcttgcgtccctccccggtttcctttgcgctcccgccttccggacctgctctcgcctatcttctttggctgtcggtgcgattcgtcaggcagcggccttgtcgaatctcgaccccaccactcgccggacccgccgacgtcccctctggagcccgccgaaacccgccgcgtctgttgaaatggccagccgcccagccgcatcctctcccgtcgaagcgcgggccccggttgggggacaggaggccggcggccccagcgcagccacccagggggaggccgccggggcccctctcgcccacggccaccacgtgtactgccagcgagtcaatggcgtgatggtgctttccaacaagacgcccgggtccgcgtcctaccgcatcagcgatagcaactttgtccaatgtggttccaactgcaccatgatcatagacggagacgtggtgcgcgggcgcccccaggacccgggggccgcggcatcccccgctcccttcgttgcggtgacaaacatcggagccggcagcgacggcgggaccgccgtcgtggcattcgggggaaccccacgtcgctcggcggggacgtctaccggtacccagacgaccgacgtccccaccgaggcccttgggggcccccctcctcctccccgcttcaccctgggtggcggctgttgttcctgtcgcgacacacggcgccgctctgcggtattcgggggggagggggatcccgtcggccccgcggagttcgtctcggacgaccggtcgtccgattccgactcggatgactcggaggacaccgactcggagacgctgtcacacgcctcctcggacgtgtccggcggggccacgtacgacgacgcccttgactccgattcgtcatcggatgactccctgcagatagatggccccgtgtgtcgcccgtggagcaatgacaccgcgcccctggatgtttgccccgggacccccggcccgggcgccgacgccggtggtccctcagcggtagacccacacgcaccgacgccaggggccggcgctggtcttgcggccgatcccgccgtggcccgggacgacgcggaggggctttcggacccccggccacgtctgggaacgggcacggcctaccccgtccccctggaactcacgcccgagaacgcggaggccgtggcgcgctttctgggagatgccgtgaaccgcgaacccgcgctcatgctggagtacttttgccggtgcgcccgcgaggaaaccaagcgtgtcccccccaggacattctgcagcccccctcgcctcacggaggacgactttgggcttctcaactacgcgctcgtggagatgcagcgcctgtgtctggacgttcctccggtcccgccgaacgcatacatgccctattatctcagggagtatgtgacgcggctggtcaacgggttcaagccgctggtgagccggtccgctcgcctttaccgcatcctgggggttctggtgcacctgcggatccggacccgggaggctagagcggccgcatcgaatataacttcgtataatgtatgctatacgaagttatccatggttgatcccgtcgttttacaacgtcgtgactgggaaaaccctggcgttacccaacttaatcgccttgcagcacatccccctttcgccagctggcgtaatagcgaagaggcccgcaccgatcgcccttcccaacagttgcgcagcctgaatggcgaatggcgctttgcctggtttccggcaccagaagcggtgccggaaagctggctggagtgcgatcttcctgaggccgatactgtcgtcgtcccctcaaactggcagatgcacggttacgatgcgcccatctacaccaacgtgacctatcccattacggtcaatccgccgtttgttcccacggagaatccgacgggttgttactcgctcacatttaatgttgatgaaagctggctacaggaaggccagacgcgaattatttttgatggcgttaactcggcgtttcatctgtggtgcaacgggcgctgggtcggttacggccaggacagtcgtttgccgtctgaatttgacctgagcgcatttttacgcgccggagaaaaccgcctcgcggtgatggtgctgcgctggagtgacggcagttatctggaagatcaggatatgtggcggatgagcggcattttccgtgacgtctcgttgctgcataaaccgactacacaaatcagcgatttccatgttgccactcgctttaatgatgatttcagccgcgctgtactggaggctgaagttcagatgtgcggcgagttgcgtgactacctacgggtaacagtttctttatggcagggtgaaacgcaggtcgccagcggcaccgcgcctttcggcggtgaaattatcgatgagcgtggtggttatgccgatcgcgtcacactacgtctgaacgtcgaaaacccgaaactgtggagcgccgaaatcccgaatctctatcgtgcggtggttgaactgcacaccgccgacggcacgctgattgaagcagaagcctgcgatgtcggtttccgcgaggtgcggattgaaaatggtctgctgctgctgaacggcaagccgttgctgattcgaggcgttaaccgtcacgagcatcatcctctgcatggtcaggtcatggatgagcagacgatggtgcaggatatcctgctgatgaagcagaacaactttaacgccgtgcgctgttcgcattatccgaaccatccgctgtggtacacgctgtgcgaccgctacggcctgtatgtggtggatgaagccaatattgaaacccacggcatggtgccaatgaatcgtctgaccgatgatccgcgctggctaccggcgatgagcgaacgcgtaacgcgaatggtgcagcgcgatcgtaatcacccgagtgtgatcatctggtcgctggggaatgaatcaggccacggcgctaatcacgacgcgctgtatcgctggatcaaatctgtcgatccttcccgcccggtgcagtatgaaggcggcggagccgacaccacggccaccgatattatttgcccgatgtacgcgcgcgtggatgaagaccagcccttcccggctgtgccgaaatggtccatcaaaaaatggctttcgctacctggagagacgcgcccgctgatcctttgcgaatacgcccacgcgatgggtaacagtcttggcggtttcgctaaatactggcaggcgtttcgtcagtatccccgtttacagggcggcttcgtctgggactgggtggatcagtcgctgattaaatatgatgaaaacggcaacccgtggtcggcttacggcggtgattttggcgatacgccgaacgatcgccagttctgtatgaacggtctggtctttgccgaccgcacgccgcatccagcgctgacggaagcaaaacaccagcagcagtttttccagttccgtttatccgggcaaaccatcgaagtgaccagcgaatacctgttccgtcatagcgataacgagctcctgcactggatggtggcgctggatggtaagccgctggcaagcggtgaagtgcctctggatgtcgctccacaaggtaaacagttgattgaactgcctgaactaccgcagccggagagcgccgggcaactctggctcacagtacgcgtagtgcaaccgaacgcgaccgcatggtcagaagccgggcacatcagcgcctggcagcagtggcgtctggcggaaaacctcagtgtgacgctccccgccgcgtcccacgccatcccgcatctgaccaccagcgaaatggatttttgcatcgagctgggtaataagcgttggcaatttaaccgccagtcaggctctctttcacagatgtggattggcgataaaaaccaactgctgacgccgctgcgcgatcagttcacccgtgcaccgctggataacgacattggcgtaagtgaagcgacccgcattgaccctaacgcctgggtcgaacgctggaaggcggcgggccattaccaggccgaagcagcgttgttgcagtgcacggcagatacacttgctgatgcggtgctgattacgaccgctcacgcgtggcagcatcaggggaaaaccttatttatcagccggaaaacctaccggattgatggtagtggtcaaatggcgattaccgttgatgttgaagtggcgagcgatacaccgcatccggcgcggattggcctgaactgccagctggcgcaggtagcagagcgggtaaactggctcggattagggccgcaagaaaactatcccgaccgccttactgccgcctgttttgaccgctgggatctgccattgtcagacatgtataccccgtacgtcttcccgagcgaaaacggtctgcgctgcgggacgcgcgaattgaattatggcccacaccagtggcgcggcgacttccagttcaacatcagccgctacagtcaacagcaactgatggaaaccagccatcgccatctgctgcacgcggaagaaggcacatggctgaatatcgacggtttccatatggggattggtggcgacgactcctggagcccgtcagtatcggcggaattccagctgagcgccggtcgctaccattaccagttggtctggtgtcaaaaaaagggcgaattcggtaagcctatccctaaccctctcctcggtctcgattctacgcgtaccgggtgctacgagatttcgattccaccgccgccttctatgaaaggttgggcttcggaatcgttttccgggacgccggctggatgatcctccagcgcggggatctcatgctggagttcttcgcccaccccaacttgtttattgcagcttataatggttacaaataaagcaatagcatcacaaatttcacaaataaagcatttttttcactgcattctagttgtggtttgtccaaactcatcaatgtatcttatcatgtctgtataccgtcgaggctggttctttccgcctcagaagccatagagcccaccgcatccccagcatgcctgctattgtcttcccaatcctcccccttgctgtcctgccccaccccaccccccagaatagaatgacacctactcagacaatgcgatgcaatttcctcattttattaggaaaggacagtgggagtggcaccttccagggtcaaggaaggcacgggggaggggcaaacaacagatggctggcaactagaaggcacagtcgaggctgatcagcgggtttaaactcaatggtgatggtgatgatgaccggtatgcatattcagatcctcttctgagatgagtttttgttcgaaccgcggaagcggccgctatcatgtgtagtgcagtttcacgcccttcagcacgggctcagaatcgtcctcgtcgaacttgcagcagctgccacagctacaacagcccttcaggcagctacagcagctggtcatgcaacacagcatgattgtgaccatcacgatggcaatcagtccggcgataaagcccagccagatgtaccagggccacttgatgtactgctcgtacttccccagttcttgcaggtcgatcaggctctcgttcagattcttggccacctcgttcagccggtcgatctctttctggatgttcacgacgctggcattgattccgctgatatcgcccaggtccacgtcggggcttgtgtggttcttaaagtacttgtccagttcctctttgaagctgtccagctcgggctgcagagggtcgtacacggtattgttcacaatgccgatcacgacgtcgcagttgccagacacgaaggtgttgtcggtggtgatgatctggggctcgtagaagttccgctgtgtcacgaaccaatgggtgccgttggacacgaacacgccttctctaggaaagtgggctttgccgtcgtggcagatggctggagcggtggtgaaattcttctcttgagcgggcacatatgtcacgtgcagaaacaccacgccgtgaggggcagactgagggaagctcatcaggtggtagcccttgccgcaaaagtccactctcttgctctggcccagcacacactcagacatcttggtggcggccagattggcagaggctctaatctcggcggctctgatcagctgctgggtcacgtatgtctggaggctctgcagtctgcctgtgatcagtctgtcgatctgcacctcggcctcaggagggtccagtctgctcaggatatcgttcagcacagagctgatggcgccgaagttggaggacagctgcttgaccagggtgttcagtgcctgggcattctggttgaccacgtcctgcagctttcccagggcgcttgctgtgctgctcaggctgtcctggatcttgccgatggcgctgttgaactggttggcgatcagcttctggttctcgtacagcacattctgggtcactccgatgccgttgaaccggtaggccatctgcatagcaaaggggatctgcagagcggcgccagctccaaatgtccagccgcttgtgattgtgccggccagcagggcagatgtgtactgggcgatcatctcatcggtcagcagaggaggcagcactgtcagtccgttaaacttctgggcgcaaatcagatccctggcggcaatgtcgcccagacaatcgccatactgcttgatgaagccggcgtcggccagtgtcactttgttgaacagcaggtcctcgatgaagctccgcttgctgggcttgctaggatcgggcagaatctggctgaaattgaagccgccgaagtccttgataggaggggtcttgtagatctgcttcacttgggcgaacacctcttgggtgttcttgtcctgttccacggcgatccctgtcagggctctattcagctgggtgcagaagctgccgtactgcagcagcaggttggagcactcggtggaatcgccgcagatgtacatggtgcagtccacgctggtcttggtcatggacacaggcaggatctctgtggtcacgctgatggtgaagttggtggggatagcgatagagttgttggagtaggccacgctgttctcggcgcccagagacattgtgtaggcaatgatgctctggctggccacagatctggcccgtctggggctgtttgtctgtgtctggtagctggcacagatgccagcgccgatggggatgtcgcactcgtagctattgttcacgtgctcggctccgatcagacagccggctctggtctgaaacacattgctgccggtggagtacacccgccatgtaggtgtcagctgatcggcgtgaatggccacgggcacttcggtacagttcacgtcctggtacagcactgccacctgattgctggtgttggtgccaggggtgatcacagacactccgccgaagctgcaaggggtgatgtccaggatttccagtgtctggggatctctaacggcgtctgtggtatcggcgatatcccggccaaactgctggaatggcaggaacttcttgttgctctctgtcagcacgccggtgccggtcaggccgttgaagttgaagttcacgcatttgttcttcacgagattggtgcttttcttagggccgcacactgtggcaggggcatgcagcagttcgaagctcagcaccaccactctgtagggctgatagcccacgccatttgtgggctgaaagccgtaggactgcagtgggaagtagcagttgaagccttccacgccgttacaaggggtgctgccggcctgatagatctcggtggagatgtcccgctcgaagggcttcagattggacttccggaacagccggtacaggtaattgtagttgccgccgactttggagtccaggttgttgctgttccaggcaatcacacagccggtgaagtcgtcgggcagcttgtagttgtagtcggcgatcttgcctgtctgtccaggggcaatctgccgcacttcatctccccggatcacgaagctgtcggcgtacacgtttgtgaagcacaggtcgttcagcttggtaggggacacgccgtagcacttgaaggtgctgaagctggcggagttgtacagcacggagtagtcggccacgcaattgctgatccgcttccggttccaggcgtacacagaggcgaatctggtggcattgaacacctcgccgaaggggcacagattggtgatattggggaaccgcacgatggattcggtgggctgcacccggaagttgctggtctggtagatgcccttttccacggtgaaggacttcagggtgcactttgtctcgctcagaggatcaagggcacaatccacggcgtcggtgatggtgccgttctcgttgtacttcagcaggaaggttctaggctgcaggtagcccacatagtaagcggcggcaccagctgtccatccgctgctgctatcgccaggtgtcaggtagcttctgtgcagggccagcagtgtctgaaaccgggtgatgttgatgccgatgggcagatccaccaggggttccagagcagagaagccctgaggcagatcccgcacgaggttgataggggtgtgcttgctgtagatcttgaagtagccgtcgatgttcttgaacacgaactcgcgcaggttcttgaagttgccctgcttgccttccaggtccatcaggaaaggctgggacacgtactcgaaggtgcagttgttggcgctgctgtacacccggaactcgctttccatccagctcttgttgttcttgtggtagtagacgcccaggaaggggtcgttgcagaactggaactcgcacactttgatgaccacgttggtggcgttgttcacgatcagcaggctctgggtcttgctgtccagtgtggtgccgaagatccagcctctgatgatgttggacttctcggtgctggcaaagtacaccccgtcgttgaagggcagcacggggttgtcgaatctcttggtgccattggtgccggacacgtggatggcgtggaaccaggtcacgttgctgaagaaaggcaggaacaggtcctgggtagagtgcagcacgctggatctgaacaccttgtcggggtagtacacgcctctggtaaagctgttggtgtaggctggaggcagctgtgttctggtggtcaggttcacacactggctggacaccagaggcagcagcaccagaaacacgaacatggtggcggatccggatccgagctcggtaccaagcttaactagccagcttgggtctccctatagtgagtcgtattaatttcgataagccagtaagcagtgggttctctagttagccagagagctctgcttatatagacctcccaccgtacacgcctaccgcccatttgcgtcaatggggcggagttgttacgacattttggaaagtcccgttgattttggtgccaaaacaaactcccattgacgtcaatggggtggagacttggaaatccccgtgagtcaaaccgctatccacgcccattgatgtactgccaaaaccgcatcaccatggtaatagcgatgactaatacgtagatgtactgccaagtaggaaagtcccataaggtcatgtactgggcataatgccaggcgggccatttaccgtcattgacgtcaatagggggcgtacttggcatatgatacacttgatgtactgccaagtgggcagtttaccgtaaatactccacccattgacgtcaatggaaagtccctattggcgttactatgggaacatacgtcattattgacgtcaatgggcgggggtcgttgggcggtcagccaggcgggccatttaccgtaagttatgtaacgcggaactccatatatgggctatgaactaatgaccccgtaattgattactattaataactagtcaataatcaatgtcaacgcgtatatctggcccgtacatcgcctgtcgacatttaaatgctagcggtacccttaagcctgcaggactagtactgatccgaagttcctatactttctagagaataggaacttccntcgaggtcatggggttcggcgagcagatacccatccaggagctggcctatggcattgtgcgcagtgcggccacgaccgggagccccttcgtcatgttcaaagacgcggtgaaccgccactacatctacgacacccagggggcggccatcgccggctccaacctc

SEQ ID NO: 31 - DNA, 1450 bp, synthetic construct
  source 1..1450: mol_type = other DNA
agcgagttagacaggcaagcactactcgcctctgcacgcacatgcttgcctgtcaaactctaccaccccggcacgctctctgtctccatggcccgccgccgccgccatcgcggcccccgccgcccccggccgcccgggcccacgggcgccgtcccaaccgcacagtcccaggtaacctccacgcccaactcggaacccgcggtcaggagcgcgcccgcggccgccccgccgccgccccccgccagtgggcccccgccttcttgttcgctgctgctgcgccagtggctccacgttcccgagtccgcgtccgacgacgacgatgacgacgactggccggacagccccccgcccgagccggcgccagaggcccggcccaccgccgccgccccccgcccccggtccccaccgcccggcgcgggcccggggggcggggctaacccctcccaccccccctcacgccccttccgccttccgccgcgcctcgccctccgcctgcgcgtcaccgcagagcacctggcgcgcctgcgcctgcgacgcgcgggcggggagggggcgccggagccccccgcgacccccgcgacccccgcgacccccgcgacccccgcgacccccgcgcgggtgcgcttctcgccccacgtccgggtgcgccacctggtggtctgggcctcggccgcccgcctggcgcgccgcggctcgtgggcccgcgagcgggccgaccgggctcggttccggcgccgggtggcggaggccgaggcggtcatcgggccgtgcctggggcccgaggcccgtgcccgggccctggcccgcggagccggcccggcgaactcggtctaacgttacacccgaggcggcctgggtcttccgcggagctcccgggagctccgcaccaagccgctctccggagagacgatggcaggagccgcgcatatatacgctgggagccggcccgcccccgaggcgggcccgccctcggagggcgggactggccaatcggcggccgccagcgcggcggggcccggccaaccagcgtccgccgagtcttcggggcccggcccactgggcgggagttaccgcccagtgggccgggccgcccacttcccggtatggtaattaaaaacttacaagaggccttgttccgcttcccggtatggtaattagaaactcattaatgggcggccccggccgcccttcccgcttccggcaattcccgcggcccttaatgggcaaccccggtattccccgcctcccgcgccgcgcgtaaccactcccctggggttccgggttatgctaattgcttttttggcggaacacacggcccctcgcgcattggcccgcgggtcgctcaatgaacccgcattggtcccctggggttccgggtatggtaatgagtttcttcgggaaggcgggaagccccggggcaccgacgcaggccaagcccctgttgcgtcgg

SEQ ID NO: 32 - DNA, 707 bp, synthetic construct
  source 1..707: mol_type = other DNA
attatcaccccgttgcgggggtccggagatcatgcgcgggtgtcctcgaggtgcgtgaacacctctggggtgcatgccggcggacggcacgccttttaagtaaacatctgggtcgcccggcccaactggggccgggggttgggtctggctcatctcgagagccacgggggggaaccaccctccgcccagagactcgggtgatggtcgtacccgggactcaacgggttaccggattacggggactgtcggtcacggtcccgccggttcttcgatgtgccacacccaaggatgcgttgggggcgatttcgggcagcagcccgggagagcgcagcaggggacgctccgggtcgtgcacggcggttctggccgcctcccggtcctcacgcccccttttattgatctcatcgcgtacgtcggcgtacgtcctgggcccaacccgcatggtgtccaggaaggtgtccgccatttccagggcccacgacatgctcccccccgacgagcaggaagcggtccacgcaacggtcgccgccggtcgcctcgacgaggacgttcctcctgcgggaaggcacgaacgcgggtgagccccctcctccgcccccgcgtcccccctcctccgcccccgcgtcccccctcctccgcccccgcgtcccccctcctccgcccccgcgtcccccctcctccgcccccgcgtcccccctcctccgccc